European Patent Application EP 4 756 036 A2, published June 10, 2026. Title: FLOW CELLS AND METHODS. Applicant: Illumina, Inc. Application US. The sequence listing filed with the application follows.

SEQUENCE LISTING (11 sequences)

SEQ ID NO: 1 - DNA, 29 bp, synthetic construct
  source 1..29: mol_type = other DNA
  modified_base 23: mod_base = OTHER; note = Uracil
aatgatacggcgaccaccgagatctacac

SEQ ID NO: 2 - DNA, 29 bp, synthetic construct
  source 1..29: mol_type = other DNA
  modified_base 23: mod_base = i
aatgatacggcgaccaccgaganctacac

SEQ ID NO: 3 - DNA, 29 bp, synthetic construct
  source 1..29: mol_type = other DNA
  modified_base 23: mod_base = OTHER; note = alkene-thymidine
aatgatacggcgaccaccgaganctacac

SEQ ID NO: 4 - DNA, 24 bp, synthetic construct
  source 1..24: mol_type = other DNA
  modified_base 22: mod_base = OTHER; note = 8-oxoguanine
caagcagaagacggcatacganat

SEQ ID NO: 5 - DNA, 24 bp, synthetic construct
  source 1..24: mol_type = other DNA
  modified_base 20: mod_base = OTHER; note = 8-oxoguanine
caagcagaagacggcatacnagat

SEQ ID NO: 6 - DNA, 24 bp, synthetic construct
  source 1..24: mol_type = other DNA
  modified_base 20: mod_base = OTHER; note = 8-oxoguanine
  modified_base 22: mod_base = OTHER; note = 8-oxoguanine
caagcagaagacggcatacnanat

SEQ ID NO: 7 - DNA, 29 bp, synthetic construct
  source 1..29: mol_type = other DNA
  modified_base 23: mod_base = OTHER; note = allyl-T
aatgatacggcgaccaccgaganctacac

SEQ ID NO: 8 - DNA, 35 bp, synthetic construct
  source 1..35: mol_type = other DNA
gctggcacgtccgaacgcttcgttaatccgttgag

SEQ ID NO: 9 - DNA, 35 bp, synthetic construct
  source 1..35: mol_type = other DNA
cgtcgtctgccatggcgcttcggtggatatgaact

SEQ ID NO: 10 - DNA, 35 bp, synthetic construct
  source 1..35: mol_type = other DNA
acggccgctaatatcaacgcgtcgaatccgcaact

SEQ ID NO: 11 - DNA, 34 bp, synthetic construct
  source 1..34: mol_type = other DNA
gccgcgttacgttagccggactattcgatgcagc